European Patent Specification EP 3 634 584 B1, published September 18, 2024. Title: UTILIZATION OF CD39 AND CD103 FOR IDENTIFICATION OF HUMAN TUMOR REACTIVE T CELLS FOR TREATMENT OF CANCER. Applicant: Providence Health & Services - Oregon AgonOx, Inc. The sequence listing filed with the application follows.

SEQUENCE LISTING (30 sequences)

SEQ ID NO: 1 - DNA, 87 bp, Homo sapiens
ccgctcaggctggagttggctgctccctcccagacatctgtgtacttctgtgccagcagttggggtggcgagcagtacttcgggccg

SEQ ID NO: 2 - DNA, 87 bp, Homo sapiens
ctgagctctctggagctgggggactcagctttgtatttctgtgccagcagcgggacagttaacaccggggagctgttttttggagaa

SEQ ID NO: 3 - DNA, 87 bp, Homo sapiens
gagtccgccagcaccaaccagacatctatgtacctctgtgccagcagtttccgggacagggggcttcagccccagcattttggtgat

SEQ ID NO: 4 - DNA, 87 bp, Homo sapiens
acgatccagcgcacacagcaggaggactcggccgtgtatctctgtgccagcagctcgacagggggctacgagcagtacttcgggccg

SEQ ID NO: 5 - DNA, 87 bp, Homo sapiens
ctgagctctctggagctgggggactcagctttgtatttctgtgccagcagcttcggacagggggcctacgagcagtacttcgggccg

SEQ ID NO: 6 - DNA, 87 bp, Homo sapiens
cagcgcacagagcagggggactcggccatgtatctctgtgccagcaggcaggagacagccgggaacactgaagctttctttggacaa

SEQ ID NO: 7 - DNA, 87 bp, Homo sapiens
ctggagtccgccagcaccaaccagacatctatgtacctctgtgccagcagtttagctagaaacaccggggagctgttttttggagaa

SEQ ID NO: 8 - DNA, 87 bp, Homo sapiens
aagatccagcctgcaaagcttgaggactcggccgtgtatctctgtgccagcagcacgactagttcagatacgcagtattttggccca

SEQ ID NO: 9 - DNA, 87 bp, Homo sapiens
cagcgcacagagcagcgggactcggccatgtatcgctgtgccagcagcgaggagcccgggatcgatgaaaaactgttttttggcagt

SEQ ID NO: 10 - DNA, 87 bp, Homo sapiens
gagtcgcccagccccaaccagacctctctgtacttctgtgccagcagtctcgggggatatagcaatcagccccagcattttggtgat

SEQ ID NO: 11 - DNA, 87 bp, Homo sapiens
actctgacagtgaccagtgcccatcctgaagacagcagcttctacatctgcagcgcttggacaggctacgagcagtacttcgggccg

SEQ ID NO: 12 - DNA, 87 bp, Homo sapiens
atccagcgcacacagcaggaggactccgccgtgtatctctgtgccagcacccaactattaatgatcaatgagcagttcttcgggcca

SEQ ID NO: 13 - DNA, 87 bp, Homo sapiens
cgcacagagcagggggactcggccatgtatctctgtgccagcagttatggccccgggacagttaatgaaaaactgttttttggcagt

SEQ ID NO: 14 - DNA, 87 bp, Homo sapiens
ctggagtcggctgctccctcccagacatctgtgtacttctgtgccagcaagggcccctttgggcggaatgagcagttcttcgggcca

SEQ ID NO: 15 - DNA, 87 bp, Homo sapiens
atccagcgcacagagcagggggactcggccatgtatctctgtgccagcagctcgattctcggggcggggacgcagtattttggccca

SEQ ID NO: 16 - DNA, 87 bp, Homo sapiens
cgcacagagcagggggactcggccatgtatctctgtgccagcagccgcactcaggggtcgggtaaggagccccagcattttggtgat

SEQ ID NO: 17 - DNA, 87 bp, Homo sapiens
tctaagaagctccttctcagtgactctggcttctatctctgtgcctggagtgtgggactccagaacactgaagctttctttggacaa

SEQ ID NO: 18 - DNA, 87 bp, Homo sapiens
ctgagctctctggagctgggggactcagctttgtatttctgtgccagcagcgaagggtatccgtcagaaaaactgttttttggcagt

SEQ ID NO: 19 - DNA, 87 bp, Homo sapiens
aagatccggtccacaaagctggaggactcagccatgtacttctgtgccagaaacaggggtaaggggaatgagcagttcttcgggcca

SEQ ID NO: 20 - DNA, 87 bp, Homo sapiens; identical to SEQ ID NO: 1

SEQ ID NO: 21 - DNA, 87 bp, Homo sapiens
actgtgacatcggcccaaaagaacccgacagctttctatctctgtgccagcaacccagggtggtacactgaagctttctttggacaa

SEQ ID NO: 22 - DNA, 87 bp, Homo sapiens
atccagccctcagaacccagggactcagctgtgtacttctgtgccagcagcccgcgggggtcttacaatgagcagttcttcgggcca

SEQ ID NO: 23 - DNA, 87 bp, Homo sapiens
cagcgcacagagcagggggactcggccatgtatctctgtgccagcagctccccgggtagctcctacaatgagcagttcttcgggcca

SEQ ID NO: 24 - DNA, 87 bp, Homo sapiens
atcaattccctggagcttggtgactctgctgtgtatttctgtgccagcagctttggacagggggcctacgagcagtacttcgggccg

SEQ ID NO: 25 - DNA, 87 bp, Homo sapiens
aagaagctccttctcagtgactctggcttctatctctgtgcccttatactagtcgggacaatacgagagacccagtacttcgggcca

SEQ ID NO: 26 - DNA, 87 bp, Homo sapiens; identical to SEQ ID NO: 10

SEQ ID NO: 27 - DNA, 87 bp, Homo sapiens
actgtgacatcggcccaaaagaacccgacagctttctatctctgtgccagtattagtgggtggggcactgaagctttctttggacaa

SEQ ID NO: 28 - DNA, 87 bp, Homo sapiens; identical to SEQ ID NO: 13

SEQ ID NO: 29 - DNA, 87 bp, Homo sapiens
gcccaaaagaacccgacagctttctatctctgtgccagtagtcccccccgacaggggtcgcggcaagagacccagtacttcgggcca

SEQ ID NO: 30 - DNA, 87 bp, Homo sapiens
ctaaacctgagctctctggagctgggggactcagctttgtatttctgtgccagcagcggacagggggcgaagcagtacttcgggccg